European Patent Application EP 4 364 752 A1, published May 8, 2024. Title: Improved Vaccine. Applicant: OncoDNA. The sequence listing filed with the application follows.

SEQUENCE LISTING (63 sequences)

SEQ ID NO: 1 - DNA, 487 bp, synthetic construct
  source 1..487: mol_type = other DNA
  variation 159..161: product = epitope
  5'UTR 1..15: function = T7 RNA Polymerase
  5'UTR 16..65: function = 5' translation enhancer
  CDS 66..158: function = Endosomial Signal; protein_id = 62; translation = MAAPGSARRPLLLLLLLLLLGLMHCASAAMD
  3'UTR 285..419: function = Translation enhancer/mRNA stability
  CDS 162..284: function = Sequence for presentation to T lymphocytes; protein_id = 63; translation = SSDYTIVLPVIGAIVVGLCLMGMGVYKIRLRCQSSGYQRI
  variation 18: note = A or G
taatacgactcactatagggataatacatttgcttctgacacaactgtgttcactagcaacctcaatggcggcccccggcagcgcccggcgacccctgctgctgctactgctgttgctgctgctcggcctcatgcattgtgcgtcagcagcaatggacnnntcgtctgactacacaattgtgcttcctgtgattggggccatcgtggttggtctctgccttatgggtatgggtgtctataaaatccgcctaaggtgtcaatcatctggataccagagaatctaaagctcgctttcttgctgtccaatttctattaaaggttcctttgttccctaagtccaactactaaactgggggatattatgaagggccttgagcatctggattctgcctaataaaaaacatttattttcattgcaaaaaaaaaaaaaaaaaaaaaaaaaaaaaaaaaaaaaaaaaaaaaaaaaaaaaaaaaaaaaaaaaaaaaa

SEQ ID NO: 2 - DNA, 587 bp, synthetic construct
  source 1..587: mol_type = other DNA
taatacgactcactatagggataatacatttgcttctgacacaactgtgttcactagcaacctcaatggcggcccccggcagcgcccggcgacccctgctgctgctactgctgttgctgctgctcggcctcatgcattgtgcgtcagcagcaatggacccgcgactcgttcctggttggaccaagcccattacgatcggttctcatgcgcatggtgatcaagtgggccaaggtggagaatgtctgactacacaattgtgcttcctgtgattggggccatcgtggttggtcgattggggccatcgtggttggtctctgccttatgggtatgggtgtctataaaatccgcctaaggtgtcaatcatctggataccagagaatctaaagctcgctttcttgctgtccaatttctattaaaggttcctttgttccctaagtccaactactaaactgggggatattatgaagggccttgagcatctggattctgcctaataaaaaacatttattttcattgcaaaaaaaaaaaaaaaaaaaaaaaaaaaaaaaaaaaaaaaaaaaaaaaaaaaaaaaaaaaaaaaaaaaaaa

SEQ ID NO: 3 - DNA, 587 bp, synthetic construct
  source 1..587: mol_type = other DNA
taatacgactcactatagggataatacatttgcttctgacacaactgtgttcactagcaacctcaatggcggcccccggcagcgcccggcgacccctgctgctgctactgctgttgctgctgctcggcctcatgcattgtgcgtcagcagcaatggacgaggctgcacttttcggaaggtttaccatcaaaagcgatgtatggtcattccggatacttctgacagagctcattactaaatgtctgactacacaattgtgcttcctgtgattggggccatcgtggttggtcgattggggccatcgtggttggtctctgccttatgggtatgggtgtctataaaatccgcctaaggtgtcaatcatctggataccagagaatctaaagctcgctttcttgctgtccaatttctattaaaggttcctttgttccctaagtccaactactaaactgggggatattatgaagggccttgagcatctggattctgcctaataaaaaacatttattttcattgcaaaaaaaaaaaaaaaaaaaaaaaaaaaaaaaaaaaaaaaaaaaaaaaaaaaaaaaaaaaaaaaaaaaaaa

SEQ ID NO: 4 - DNA, 587 bp, synthetic construct
  source 1..587: mol_type = other DNA
taatacgactcactatagggataatacatttgcttctgacacaactgtgttcactagcaacctcaatggcggcccccggcagcgcccggcgacccctgctgctgctactgctgttgctgctgctcggcctcatgcattgtgcgtcagcagcaatggacattgacttcgtattgtctaatgcaaggccggtcttgggtgttggaggggctgcaatgcttgggatagcaacgctcgctgtgtgtctgactacacaattgtgcttcctgtgattggggccatcgtggttggtcgattggggccatcgtggttggtctctgccttatgggtatgggtgtctataaaatccgcctaaggtgtcaatcatctggataccagagaatctaaagctcgctttcttgctgtccaatttctattaaaggttcctttgttccctaagtccaactactaaactgggggatattatgaagggccttgagcatctggattctgcctaataaaaaacatttattttcattgcaaaaaaaaaaaaaaaaaaaaaaaaaaaaaaaaaaaaaaaaaaaaaaaaaaaaaaaaaaaaaaaaaaaaaa

SEQ ID NO: 5 - DNA, 587 bp, synthetic construct
  source 1..587: mol_type = other DNA
taatacgactcactatagggataatacatttgcttctgacacaactgtgttcactagcaacctcaatggcggcccccggcagcgcccggcgacccctgctgctgctactgctgttgctgctgctcggcctcatgcattgtgcgtcagcagcaatggacagacaacacagggatcgggatagagaaaaggaaagagaaaaagagaagggtaagccgaaaccgagatcacctcaaccactctgtctgactacacaattgtgcttcctgtgattggggccatcgtggttggtcgattggggccatcgtggttggtctctgccttatgggtatgggtgtctataaaatccgcctaaggtgtcaatcatctggataccagagaatctaaagctcgctttcttgctgtccaatttctattaaaggttcctttgttccctaagtccaactactaaactgggggatattatgaagggccttgagcatctggattctgcctaataaaaaacatttattttcattgcaaaaaaaaaaaaaaaaaaaaaaaaaaaaaaaaaaaaaaaaaaaaaaaaaaaaaaaaaaaaaaaaaaaaaa

SEQ ID NO: 6 - DNA, 587 bp, synthetic construct
  source 1..587: mol_type = other DNA
taatacgactcactatagggataatacatttgcttctgacacaactgtgttcactagcaacctcaatggcggcccccggcagcgcccggcgacccctgctgctgctactgctgttgctgctgctcggcctcatgcattgtgcgtcagcagcaatggacaagcaacaagaggtacagttcaaatcatattacctgccaaaagatgatgagtattatcaattttgttatgtggacgaggactgtctgactacacaattgtgcttcctgtgattggggccatcgtggttggtcgattggggccatcgtggttggtctctgccttatgggtatgggtgtctataaaatccgcctaaggtgtcaatcatctggataccagagaatctaaagctcgctttcttgctgtccaatttctattaaaggttcctttgttccctaagtccaactactaaactgggggatattatgaagggccttgagcatctggattctgcctaataaaaaacatttattttcattgcaaaaaaaaaaaaaaaaaaaaaaaaaaaaaaaaaaaaaaaaaaaaaaaaaaaaaaaaaaaaaaaaaaaaaa

SEQ ID NO: 7 - DNA, 587 bp, synthetic construct
  source 1..587: mol_type = other DNA
taatacgactcactatagggataatacatttgcttctgacacaactgtgttcactagcaacctcaatggcggcccccggcagcgcccggcgacccctgctgctgctactgctgttgctgctgctcggcctcatgcattgtgcgtcagcagcaatggacgtcgtatatttcactgctatgttcccatatgtggtactggtgatcctgctcataaggggggtaacccttcctggtgcaggatgtctgactacacaattgtgcttcctgtgattggggccatcgtggttggtcgattggggccatcgtggttggtctctgccttatgggtatgggtgtctataaaatccgcctaaggtgtcaatcatctggataccagagaatctaaagctcgctttcttgctgtccaatttctattaaaggttcctttgttccctaagtccaactactaaactgggggatattatgaagggccttgagcatctggattctgcctaataaaaaacatttattttcattgcaaaaaaaaaaaaaaaaaaaaaaaaaaaaaaaaaaaaaaaaaaaaaaaaaaaaaaaaaaaaaaaaaaaaaa

SEQ ID NO: 8 - DNA, 587 bp, synthetic construct
  source 1..587: mol_type = other DNA
taatacgactcactatagggataatacatttgcttctgacacaactgtgttcactagcaacctcaatggcggcccccggcagcgcccggcgacccctgctgctgctactgctgttgctgctgctcggcctcatgcattgtgcgtcagcagcaatggacgccggggacgctcccacatttcccaggccttccggaccacgcaatactctctggcaagaactcccagccgtccaagccagctgtctgactacacaattgtgcttcctgtgattggggccatcgtggttggtcgattggggccatcgtggttggtctctgccttatgggtatgggtgtctataaaatccgcctaaggtgtcaatcatctggataccagagaatctaaagctcgctttcttgctgtccaatttctattaaaggttcctttgttccctaagtccaactactaaactgggggatattatgaagggccttgagcatctggattctgcctaataaaaaacatttattttcattgcaaaaaaaaaaaaaaaaaaaaaaaaaaaaaaaaaaaaaaaaaaaaaaaaaaaaaaaaaaaaaaaaaaaaaa

SEQ ID NO: 9 - DNA, 587 bp, synthetic construct
  source 1..587: mol_type = other DNA
taatacgactcactatagggataatacatttgcttctgacacaactgtgttcactagcaacctcaatggcggcccccggcagcgcccggcgacccctgctgctgctactgctgttgctgctgctcggcctcatgcattgtgcgtcagcagcaatggaccataatctcattgcggaagttggagcccccgcggcgctgggcgtgagaggggcccttgagggattgccacggccccccccatgtctgactacacaattgtgcttcctgtgattggggccatcgtggttggtcgattggggccatcgtggttggtctctgccttatgggtatgggtgtctataaaatccgcctaaggtgtcaatcatctggataccagagaatctaaagctcgctttcttgctgtccaatttctattaaaggttcctttgttccctaagtccaactactaaactgggggatattatgaagggccttgagcatctggattctgcctaataaaaaacatttattttcattgcaaaaaaaaaaaaaaaaaaaaaaaaaaaaaaaaaaaaaaaaaaaaaaaaaaaaaaaaaaaaaaaaaaaaaa

SEQ ID NO: 10 - DNA, 587 bp, synthetic construct
  source 1..587: mol_type = other DNA
taatacgactcactatagggataatacatttgcttctgacacaactgtgttcactagcaacctcaatggcggcccccggcagcgcccggcgacccctgctgctgctactgctgttgctgctgctcggcctcatgcattgtgcgtcagcagcaatggacaacatcccccgactggtcccaggctggaccaaaccgattactatcgggtcccatgctcatggtgaccaagtaggacaagggtgtctgactacacaattgtgcttcctgtgattggggccatcgtggttggtcgattggggccatcgtggttggtctctgccttatgggtatgggtgtctataaaatccgcctaaggtgtcaatcatctggataccagagaatctaaagctcgctttcttgctgtccaatttctattaaaggttcctttgttccctaagtccaactactaaactgggggatattatgaagggccttgagcatctggattctgcctaataaaaaacatttattttcattgcaaaaaaaaaaaaaaaaaaaaaaaaaaaaaaaaaaaaaaaaaaaaaaaaaaaaaaaaaaaaaaaaaaaaaa

SEQ ID NO: 11 - DNA, 587 bp, synthetic construct
  source 1..587: mol_type = other DNA
taatacgactcactatagggataatacatttgcttctgacacaactgtgttcactagcaacctcaatggcggcccccggcagcgcccggcgacccctgctgctgctactgctgttgctgctgctcggcctcatgcattgtgcgtcagcagcaatggactgcctgcaagactggggtccattcttctcactcgccgtgcctagtatgcttatgatctgtttcgagtggtgggcttacgagtgtctgactacacaattgtgcttcctgtgattggggccatcgtggttggtcgattggggccatcgtggttggtctctgccttatgggtatgggtgtctataaaatccgcctaaggtgtcaatcatctggataccagagaatctaaagctcgctttcttgctgtccaatttctattaaaggttcctttgttccctaagtccaactactaaactgggggatattatgaagggccttgagcatctggattctgcctaataaaaaacatttattttcattgcaaaaaaaaaaaaaaaaaaaaaaaaaaaaaaaaaaaaaaaaaaaaaaaaaaaaaaaaaaaaaaaaaaaaaa

SEQ ID NO: 12 - DNA, 587 bp, synthetic construct
  source 1..587: mol_type = other DNA
taatacgactcactatagggataatacatttgcttctgacacaactgtgttcactagcaacctcaatggcggcccccggcagcgcccggcgacccctgctgctgctactgctgttgctgctgctcggcctcatgcattgtgcgtcagcagcaatggactttgtgctcagcaacgccaggccggtcctcggcgtgggtggagctgcgatgctcggcattgccaccttggcggtgaagcggtgtctgactacacaattgtgcttcctgtgattggggccatcgtggttggtcgattggggccatcgtggttggtctctgccttatgggtatgggtgtctataaaatccgcctaaggtgtcaatcatctggataccagagaatctaaagctcgctttcttgctgtccaatttctattaaaggttcctttgttccctaagtccaactactaaactgggggatattatgaagggccttgagcatctggattctgcctaataaaaaacatttattttcattgcaaaaaaaaaaaaaaaaaaaaaaaaaaaaaaaaaaaaaaaaaaaaaaaaaaaaaaaaaaaaaaaaaaaaaa

SEQ ID NO: 13 - DNA, 587 bp, synthetic construct
  source 1..587: mol_type = other DNA
taatacgactcactatagggataatacatttgcttctgacacaactgtgttcactagcaacctcaatggcggcccccggcagcgcccggcgacccctgctgctgctactgctgttgctgctgctcggcctcatgcattgtgcgtcagcagcaatggacgccattacaagagctgagagcttttctgtcatgtatgccccctttgctactaagatccgagcagacaaaatagagaaggtctgtctgactacacaattgtgcttcctgtgattggggccatcgtggttggtcgattggggccatcgtggttggtctctgccttatgggtatgggtgtctataaaatccgcctaaggtgtcaatcatctggataccagagaatctaaagctcgctttcttgctgtccaatttctattaaaggttcctttgttccctaagtccaactactaaactgggggatattatgaagggccttgagcatctggattctgcctaataaaaaacatttattttcattgcaaaaaaaaaaaaaaaaaaaaaaaaaaaaaaaaaaaaaaaaaaaaaaaaaaaaaaaaaaaaaaaaaaaaaa

SEQ ID NO: 14 - DNA, 587 bp, synthetic construct
  source 1..587: mol_type = other DNA
taatacgactcactatagggataatacatttgcttctgacacaactgtgttcactagcaacctcaatggcggcccccggcagcgcccggcgacccctgctgctgctactgctgttgctgctgctcggcctcatgcattgtgcgtcagcagcaatggacggatggaagaccacctgtgaatactacaccttcatgtgggttaccctccccatcgacctgaacaataaatcagcgaaacaatgtctgactacacaattgtgcttcctgtgattggggccatcgtggttggtcgattggggccatcgtggttggtctctgccttatgggtatgggtgtctataaaatccgcctaaggtgtcaatcatctggataccagagaatctaaagctcgctttcttgctgtccaatttctattaaaggttcctttgttccctaagtccaactactaaactgggggatattatgaagggccttgagcatctggattctgcctaataaaaaacatttattttcattgcaaaaaaaaaaaaaaaaaaaaaaaaaaaaaaaaaaaaaaaaaaaaaaaaaaaaaaaaaaaaaaaaaaaaaa

SEQ ID NO: 15 - DNA, 587 bp, synthetic construct
  source 1..587: mol_type = other DNA
taatacgactcactatagggataatacatttgcttctgacacaactgtgttcactagcaacctcaatggcggcccccggcagcgcccggcgacccctgctgctgctactgctgttgctgctgctcggcctcatgcattgtgcgtcagcagcaatggactgggaggaatttactgatcaactgtcattcatcggaagaataaggccgttggccgaaaaaacgggcatttgcaaaatccgatgtctgactacacaattgtgcttcctgtgattggggccatcgtggttggtcgattggggccatcgtggttggtctctgccttatgggtatgggtgtctataaaatccgcctaaggtgtcaatcatctggataccagagaatctaaagctcgctttcttgctgtccaatttctattaaaggttcctttgttccctaagtccaactactaaactgggggatattatgaagggccttgagcatctggattctgcctaataaaaaacatttattttcattgcaaaaaaaaaaaaaaaaaaaaaaaaaaaaaaaaaaaaaaaaaaaaaaaaaaaaaaaaaaaaaaaaaaaaaa

SEQ ID NO: 16 - DNA, 587 bp, synthetic construct
  source 1..587: mol_type = other DNA
taatacgactcactatagggataatacatttgcttctgacacaactgtgttcactagcaacctcaatggcggcccccggcagcgcccggcgacccctgctgctgctactgctgttgctgctgctcggcctcatgcattgtgcgtcagcagcaatggaccttcccggcatcggtcatgcgtgtggtcacaatctgatagcggaggtcggtgctccagccgcacttggtgtccgaggagcctgtctgactacacaattgtgcttcctgtgattggggccatcgtggttggtcgattggggccatcgtggttggtctctgccttatgggtatgggtgtctataaaatccgcctaaggtgtcaatcatctggataccagagaatctaaagctcgctttcttgctgtccaatttctattaaaggttcctttgttccctaagtccaactactaaactgggggatattatgaagggccttgagcatctggattctgcctaataaaaaacatttattttcattgcaaaaaaaaaaaaaaaaaaaaaaaaaaaaaaaaaaaaaaaaaaaaaaaaaaaaaaaaaaaaaaaaaaaaaa

SEQ ID NO: 17 - DNA, 587 bp, synthetic construct
  source 1..587: mol_type = other DNA
taatacgactcactatagggataatacatttgcttctgacacaactgtgttcactagcaacctcaatggcggcccccggcagcgcccggcgacccctgctgctgctactgctgttgctgctgctcggcctcatgcattgtgcgtcagcagcaatggacttctcagaggacggagaatatttcgcttatggggtctcagcatcagggtccgattgggtaacgataaaatttatgaaagtttgtctgactacacaattgtgcttcctgtgattggggccatcgtggttggtcgattggggccatcgtggttggtctctgccttatgggtatgggtgtctataaaatccgcctaaggtgtcaatcatctggataccagagaatctaaagctcgctttcttgctgtccaatttctattaaaggttcctttgttccctaagtccaactactaaactgggggatattatgaagggccttgagcatctggattctgcctaataaaaaacatttattttcattgcaaaaaaaaaaaaaaaaaaaaaaaaaaaaaaaaaaaaaaaaaaaaaaaaaaaaaaaaaaaaaaaaaaaaaa

SEQ ID NO: 18 - DNA, 587 bp, synthetic construct
  source 1..587: mol_type = other DNA
taatacgactcactatagggataatacatttgcttctgacacaactgtgttcactagcaacctcaatggcggcccccggcagcgcccggcgacccctgctgctgctactgctgttgctgctgctcggcctcatgcattgtgcgtcagcagcaatggactgtggtggcggtatccagacccgcgaagtttattgcgcccaatccctcccggctgcagccgctctgagggctaaggaggtttgtctgactacacaattgtgcttcctgtgattggggccatcgtggttggtcgattggggccatcgtggttggtctctgccttatgggtatgggtgtctataaaatccgcctaaggtgtcaatcatctggataccagagaatctaaagctcgctttcttgctgtccaatttctattaaaggttcctttgttccctaagtccaactactaaactgggggatattatgaagggccttgagcatctggattctgcctaataaaaaacatttattttcattgcaaaaaaaaaaaaaaaaaaaaaaaaaaaaaaaaaaaaaaaaaaaaaaaaaaaaaaaaaaaaaaaaaaaaaa

SEQ ID NO: 19 - DNA, 587 bp, synthetic construct
  source 1..587: mol_type = other DNA
taatacgactcactatagggataatacatttgcttctgacacaactgtgttcactagcaacctcaatggcggcccccggcagcgcccggcgacccctgctgctgctactgctgttgctgctgctcggcctcatgcattgtgcgtcagcagcaatggaccccgacgctatgcttctggcggaaattcgctcagttggccagacggaatacaacgggttccacctgtccaaaaagatagtctgtctgactacacaattgtgcttcctgtgattggggccatcgtggttggtcgattggggccatcgtggttggtctctgccttatgggtatgggtgtctataaaatccgcctaaggtgtcaatcatctggataccagagaatctaaagctcgctttcttgctgtccaatttctattaaaggttcctttgttccctaagtccaactactaaactgggggatattatgaagggccttgagcatctggattctgcctaataaaaaacatttattttcattgcaaaaaaaaaaaaaaaaaaaaaaaaaaaaaaaaaaaaaaaaaaaaaaaaaaaaaaaaaaaaaaaaaaaaaa

SEQ ID NO: 20 - DNA, 587 bp, synthetic construct
  source 1..587: mol_type = other DNA
taatacgactcactatagggataatacatttgcttctgacacaactgtgttcactagcaacctcaatggcggcccccggcagcgcccggcgacccctgctgctgctactgctgttgctgctgctcggcctcatgcattgtgcgtcagcagcaatggacagctccggcaagcttctcgctaaaaccgtatatctgcgggaggcggaggggatgtttgacatacacattgtacaaaacccgtgtctgactacacaattgtgcttcctgtgattggggccatcgtggttggtcgattggggccatcgtggttggtctctgccttatgggtatgggtgtctataaaatccgcctaaggtgtcaatcatctggataccagagaatctaaagctcgctttcttgctgtccaatttctattaaaggttcctttgttccctaagtccaactactaaactgggggatattatgaagggccttgagcatctggattctgcctaataaaaaacatttattttcattgcaaaaaaaaaaaaaaaaaaaaaaaaaaaaaaaaaaaaaaaaaaaaaaaaaaaaaaaaaaaaaaaaaaaaaa

SEQ ID NO: 21 - DNA, 587 bp, synthetic construct
  source 1..587: mol_type = other DNA
taatacgactcactatagggataatacatttgcttctgacacaactgtgttcactagcaacctcaatggcggcccccggcagcgcccggcgacccctgctgctgctactgctgttgctgctgctcggcctcatgcattgtgcgtcagcagcaatggacagcgtacccggcgcggtgcttatggacattaagtcagagcttttgaggtatgagatacagttcaaaggcaatgcacacacatgtctgactacacaattgtgcttcctgtgattggggccatcgtggttggtcgattggggccatcgtggttggtctctgccttatgggtatgggtgtctataaaatccgcctaaggtgtcaatcatctggataccagagaatctaaagctcgctttcttgctgtccaatttctattaaaggttcctttgttccctaagtccaactactaaactgggggatattatgaagggccttgagcatctggattctgcctaataaaaaacatttattttcattgcaaaaaaaaaaaaaaaaaaaaaaaaaaaaaaaaaaaaaaaaaaaaaaaaaaaaaaaaaaaaaaaaaaaaaa

SEQ ID NO: 22 - DNA, 587 bp, synthetic construct
  source 1..587: mol_type = other DNA
taatacgactcactatagggataatacatttgcttctgacacaactgtgttcactagcaacctcaatggcggcccccggcagcgcccggcgacccctgctgctgctactgctgttgctgctgctcggcctcatgcattgtgcgtcagcagcaatggactctaaacaagaaggcttcatagacacggccctgcgaaagtacgtcgaaaacctggtgttgcatgggattcctatggcatcatgtctgactacacaattgtgcttcctgtgattggggccatcgtggttggtcgattggggccatcgtggttggtctctgccttatgggtatgggtgtctataaaatccgcctaaggtgtcaatcatctggataccagagaatctaaagctcgctttcttgctgtccaatttctattaaaggttcctttgttccctaagtccaactactaaactgggggatattatgaagggccttgagcatctggattctgcctaataaaaaacatttattttcattgcaaaaaaaaaaaaaaaaaaaaaaaaaaaaaaaaaaaaaaaaaaaaaaaaaaaaaaaaaaaaaaaaaaaaaa

SEQ ID NO: 23 - DNA, 587 bp, synthetic construct
  source 1..587: mol_type = other DNA
taatacgactcactatagggataatacatttgcttctgacacaactgtgttcactagcaacctcaatggcggcccccggcagcgcccggcgacccctgctgctgctactgctgttgctgctgctcggcctcatgcattgtgcgtcagcagcaatggacataatgaaccatgctgacagtgctacaggaaaggtcaagatagaacgggagggggtcttttacccgcttttgctgcaaagctgtctgactacacaattgtgcttcctgtgattggggccatcgtggttggtcgattggggccatcgtggttggtctctgccttatgggtatgggtgtctataaaatccgcctaaggtgtcaatcatctggataccagagaatctaaagctcgctttcttgctgtccaatttctattaaaggttcctttgttccctaagtccaactactaaactgggggatattatgaagggccttgagcatctggattctgcctaataaaaaacatttattttcattgcaaaaaaaaaaaaaaaaaaaaaaaaaaaaaaaaaaaaaaaaaaaaaaaaaaaaaaaaaaaaaaaaaaaaaa

SEQ ID NO: 24 - DNA, 587 bp, synthetic construct
  source 1..587: mol_type = other DNA
taatacgactcactatagggataatacatttgcttctgacacaactgtgttcactagcaacctcaatggcggcccccggcagcgcccggcgacccctgctgctgctactgctgttgctgctgctcggcctcatgcattgtgcgtcagcagcaatggacgcgagcccgagcaacttgaaaggcaagaccgagatcttcgctcacgtagaactgagagttatgcagggactgtatatagattgtctgactacacaattgtgcttcctgtgattggggccatcgtggttggtcgattggggccatcgtggttggtctctgccttatgggtatgggtgtctataaaatccgcctaaggtgtcaatcatctggataccagagaatctaaagctcgctttcttgctgtccaatttctattaaaggttcctttgttccctaagtccaactactaaactgggggatattatgaagggccttgagcatctggattctgcctaataaaaaacatttattttcattgcaaaaaaaaaaaaaaaaaaaaaaaaaaaaaaaaaaaaaaaaaaaaaaaaaaaaaaaaaaaaaaaaaaaaaa

SEQ ID NO: 25 - DNA, 587 bp, synthetic construct
  source 1..587: mol_type = other DNA
taatacgactcactatagggataatacatttgcttctgacacaactgtgttcactagcaacctcaatggcggcccccggcagcgcccggcgacccctgctgctgctactgctgttgctgctgctcggcctcatgcattgtgcgtcagcagcaatggacgaagctggagtaggttttttgagcaaggatcgaaagattgctctttatttgacgaatgaacaccaggtctcaatgcccatctgtctgactacacaattgtgcttcctgtgattggggccatcgtggttggtcgattggggccatcgtggttggtctctgccttatgggtatgggtgtctataaaatccgcctaaggtgtcaatcatctggataccagagaatctaaagctcgctttcttgctgtccaatttctattaaaggttcctttgttccctaagtccaactactaaactgggggatattatgaagggccttgagcatctggattctgcctaataaaaaacatttattttcattgcaaaaaaaaaaaaaaaaaaaaaaaaaaaaaaaaaaaaaaaaaaaaaaaaaaaaaaaaaaaaaaaaaaaaaa

SEQ ID NO: 26 - DNA, 587 bp, synthetic construct
  source 1..587: mol_type = other DNA
taatacgactcactatagggataatacatttgcttctgacacaactgtgttcactagcaacctcaatggcggcccccggcagcgcccggcgacccctgctgctgctactgctgttgctgctgctcggcctcatgcattgtgcgtcagcagcaatggacagtatgctcagattttataataaaggcgttaagggaccccttgaagcgagcgatactgttgaacacgcactcattcaaatatgtctgactacacaattgtgcttcctgtgattggggccatcgtggttggtcgattggggccatcgtggttggtctctgccttatgggtatgggtgtctataaaatccgcctaaggtgtcaatcatctggataccagagaatctaaagctcgctttcttgctgtccaatttctattaaaggttcctttgttccctaagtccaactactaaactgggggatattatgaagggccttgagcatctggattctgcctaataaaaaacatttattttcattgcaaaaaaaaaaaaaaaaaaaaaaaaaaaaaaaaaaaaaaaaaaaaaaaaaaaaaaaaaaaaaaaaaaaaaa

SEQ ID NO: 27 - DNA, 587 bp, synthetic construct
  source 1..587: mol_type = other DNA
taatacgactcactatagggataatacatttgcttctgacacaactgtgttcactagcaacctcaatggcggcccccggcagcgcccggcgacccctgctgctgctactgctgttgctgctgctcggcctcatgcattgtgcgtcagcagcaatggacgtctttccactggaggagcagatgggaaaaataacacgagatggcagttaccatatcgcagttctcgcgaattccaagctctgtctgactacacaattgtgcttcctgtgattggggccatcgtggttggtcgattggggccatcgtggttggtctctgccttatgggtatgggtgtctataaaatccgcctaaggtgtcaatcatctggataccagagaatctaaagctcgctttcttgctgtccaatttctattaaaggttcctttgttccctaagtccaactactaaactgggggatattatgaagggccttgagcatctggattctgcctaataaaaaacatttattttcattgcaaaaaaaaaaaaaaaaaaaaaaaaaaaaaaaaaaaaaaaaaaaaaaaaaaaaaaaaaaaaaaaaaaaaaa

SEQ ID NO: 28 - DNA, 587 bp, synthetic construct
  source 1..587: mol_type = other DNA
taatacgactcactatagggataatacatttgcttctgacacaactgtgttcactagcaacctcaatggcggcccccggcagcgcccggcgacccctgctgctgctactgctgttgctgctgctcggcctcatgcattgtgcgtcagcagcaatggactccgagctctacaagagggcgggcaagatgaatacggttggtctctcacaagaagcgatactgatcgatccgtttcacgtgtgtctgactacacaattgtgcttcctgtgattggggccatcgtggttggtcgattggggccatcgtggttggtctctgccttatgggtatgggtgtctataaaatccgcctaaggtgtcaatcatctggataccagagaatctaaagctcgctttcttgctgtccaatttctattaaaggttcctttgttccctaagtccaactactaaactgggggatattatgaagggccttgagcatctggattctgcctaataaaaaacatttattttcattgcaaaaaaaaaaaaaaaaaaaaaaaaaaaaaaaaaaaaaaaaaaaaaaaaaaaaaaaaaaaaaaaaaaaaaa

SEQ ID NO: 29 - DNA, 587 bp, synthetic construct
  source 1..587: mol_type = other DNA
taatacgactcactatagggataatacatttgcttctgacacaactgtgttcactagcaacctcaatggcggcccccggcagcgcccggcgacccctgctgctgctactgctgttgctgctgctcggcctcatgcattgtgcgtcagcagcaatggactcccttctggggctgaaacagatttctccagtggatagggcagccatggagatttataacgtttttcacgggaaaacagagtgtctgactacacaattgtgcttcctgtgattggggccatcgtggttggtcgattggggccatcgtggttggtctctgccttatgggtatgggtgtctataaaatccgcctaaggtgtcaatcatctggataccagagaatctaaagctcgctttcttgctgtccaatttctattaaaggttcctttgttccctaagtccaactactaaactgggggatattatgaagggccttgagcatctggattctgcctaataaaaaacatttattttcattgcaaaaaaaaaaaaaaaaaaaaaaaaaaaaaaaaaaaaaaaaaaaaaaaaaaaaaaaaaaaaaaaaaaaaaa

SEQ ID NO: 30 - DNA, 587 bp, synthetic construct
  source 1..587: mol_type = other DNA
taatacgactcactatagggataatacatttgcttctgacacaactgtgttcactagcaacctcaatggcggcccccggcagcgcccggcgacccctgctgctgctactgctgttgctgctgctcggcctcatgcattgtgcgtcagcagcaatggacattgtaacagcgggtagaccccaccttcttgagatgttgaactcagtccaattcgctggcgagagtaaatacaaaatcgactgtctgactacacaattgtgcttcctgtgattggggccatcgtggttggtcgattggggccatcgtggttggtctctgccttatgggtatgggtgtctataaaatccgcctaaggtgtcaatcatctggataccagagaatctaaagctcgctttcttgctgtccaatttctattaaaggttcctttgttccctaagtccaactactaaactgggggatattatgaagggccttgagcatctggattctgcctaataaaaaacatttattttcattgcaaaaaaaaaaaaaaaaaaaaaaaaaaaaaaaaaaaaaaaaaaaaaaaaaaaaaaaaaaaaaaaaaaaaaa

SEQ ID NO: 31 - DNA, 587 bp, synthetic construct
  source 1..587: mol_type = other DNA
taatacgactcactatagggataatacatttgcttctgacacaactgtgttcactagcaacctcaatggcggcccccggcagcgcccggcgacccctgctgctgctactgctgttgctgctgctcggcctcatgcattgtgcgtcagcagcaatggacgtggctcacgggagcgagcaaacagaaatccccttttactctggactcgttaacattgatttggcaaaactcaaacggatgtgtctgactacacaattgtgcttcctgtgattggggccatcgtggttggtcgattggggccatcgtggttggtctctgccttatgggtatgggtgtctataaaatccgcctaaggtgtcaatcatctggataccagagaatctaaagctcgctttcttgctgtccaatttctattaaaggttcctttgttccctaagtccaactactaaactgggggatattatgaagggccttgagcatctggattctgcctaataaaaaacatttattttcattgcaaaaaaaaaaaaaaaaaaaaaaaaaaaaaaaaaaaaaaaaaaaaaaaaaaaaaaaaaaaaaaaaaaaaaa

SEQ ID NO: 32 - DNA, 587 bp, synthetic construct
  source 1..587: mol_type = other DNA
taatacgactcactatagggataatacatttgcttctgacacaactgtgttcactagcaacctcaatggcggcccccggcagcgcccggcgacccctgctgctgctactgctgttgctgctgctcggcctcatgcattgtgcgtcagcagcaatggaccagtacctctcacccatggtacatattctgggacttgagagggtggcaaagaatactgaaaaattcgccggtatatctgattgtctgactacacaattgtgcttcctgtgattggggccatcgtggttggtcgattggggccatcgtggttggtctctgccttatgggtatgggtgtctataaaatccgcctaaggtgtcaatcatctggataccagagaatctaaagctcgctttcttgctgtccaatttctattaaaggttcctttgttccctaagtccaactactaaactgggggatattatgaagggccttgagcatctggattctgcctaataaaaaacatttattttcattgcaaaaaaaaaaaaaaaaaaaaaaaaaaaaaaaaaaaaaaaaaaaaaaaaaaaaaaaaaaaaaaaaaaaaaa

SEQ ID NO: 33 - DNA, 587 bp, synthetic construct
  source 1..587: mol_type = other DNA
taatacgactcactatagggataatacatttgcttctgacacaactgtgttcactagcaacctcaatggcggcccccggcagcgcccggcgacccctgctgctgctactgctgttgctgctgctcggcctcatgcattgtgcgtcagcagcaatggacatgtcccaggttatagagatcaaaaatcgggcacttgctgggcactttaccgattatttggaaggcgtaagtaagcccctttgtctgactacacaattgtgcttcctgtgattggggccatcgtggttggtcgattggggccatcgtggttggtctctgccttatgggtatgggtgtctataaaatccgcctaaggtgtcaatcatctggataccagagaatctaaagctcgctttcttgctgtccaatttctattaaaggttcctttgttccctaagtccaactactaaactgggggatattatgaagggccttgagcatctggattctgcctaataaaaaacatttattttcattgcaaaaaaaaaaaaaaaaaaaaaaaaaaaaaaaaaaaaaaaaaaaaaaaaaaaaaaaaaaaaaaaaaaaaaa

SEQ ID NO: 34 - DNA, 587 bp, synthetic construct
  source 1..587: mol_type = other DNA
taatacgactcactatagggataatacatttgcttctgacacaactgtgttcactagcaacctcaatggcggcccccggcagcgcccggcgacccctgctgctgctactgctgttgctgctgctcggcctcatgcattgtgcgtcagcagcaatggacatgcttgcaatctctcttcgggggtatccttcaggggctgtgcacattaacaccgaggttgaacagaagttgaaggatttttgtctgactacacaattgtgcttcctgtgattggggccatcgtggttggtcgattggggccatcgtggttggtctctgccttatgggtatgggtgtctataaaatccgcctaaggtgtcaatcatctggataccagagaatctaaagctcgctttcttgctgtccaatttctattaaaggttcctttgttccctaagtccaactactaaactgggggatattatgaagggccttgagcatctggattctgcctaataaaaaacatttattttcattgcaaaaaaaaaaaaaaaaaaaaaaaaaaaaaaaaaaaaaaaaaaaaaaaaaaaaaaaaaaaaaaaaaaaaaa

SEQ ID NO: 35 - DNA, 587 bp, synthetic construct
  source 1..587: mol_type = other DNA
taatacgactcactatagggataatacatttgcttctgacacaactgtgttcactagcaacctcaatggcggcccccggcagcgcccggcgacccctgctgctgctactgctgttgctgctgctcggcctcatgcattgtgcgtcagcagcaatggacgttgagcctctttcattgttcaagaaaaatcttggctacagaacgatccagcatgctatggcagactcagaggtaattggttgtctgactacacaattgtgcttcctgtgattggggccatcgtggttggtcgattggggccatcgtggttggtctctgccttatgggtatgggtgtctataaaatccgcctaaggtgtcaatcatctggataccagagaatctaaagctcgctttcttgctgtccaatttctattaaaggttcctttgttccctaagtccaactactaaactgggggatattatgaagggccttgagcatctggattctgcctaataaaaaacatttattttcattgcaaaaaaaaaaaaaaaaaaaaaaaaaaaaaaaaaaaaaaaaaaaaaaaaaaaaaaaaaaaaaaaaaaaaaa

SEQ ID NO: 36 - DNA, 587 bp, synthetic construct
  source 1..587: mol_type = other DNA
taatacgactcactatagggataatacatttgcttctgacacaactgtgttcactagcaacctcaatggcggcccccggcagcgcccggcgacccctgctgctgctactgctgttgctgctgctcggcctcatgcattgtgcgtcagcagcaatggactcaaaggtgaaagtacttaacatcagcgaactccatggctatgagtttcaggcaatgggtacgcgagaccccgctatactttgtctgactacacaattgtgcttcctgtgattggggccatcgtggttggtcgattggggccatcgtggttggtctctgccttatgggtatgggtgtctataaaatccgcctaaggtgtcaatcatctggataccagagaatctaaagctcgctttcttgctgtccaatttctattaaaggttcctttgttccctaagtccaactactaaactgggggatattatgaagggccttgagcatctggattctgcctaataaaaaacatttattttcattgcaaaaaaaaaaaaaaaaaaaaaaaaaaaaaaaaaaaaaaaaaaaaaaaaaaaaaaaaaaaaaaaaaaaaaa

SEQ ID NO: 37 - DNA, 587 bp, synthetic construct
  source 1..587: mol_type = other DNA
taatacgactcactatagggataatacatttgcttctgacacaactgtgttcactagcaacctcaatggcggcccccggcagcgcccggcgacccctgctgctgctactgctgttgctgctgctcggcctcatgcattgtgcgtcagcagcaatggaccacaagaaactggccttgatcggaccaaaccaggatgtccgaatgacactctcaggatttgaggctagtgtagaaatctattgtctgactacacaattgtgcttcctgtgattggggccatcgtggttggtcgattggggccatcgtggttggtctctgccttatgggtatgggtgtctataaaatccgcctaaggtgtcaatcatctggataccagagaatctaaagctcgctttcttgctgtccaatttctattaaaggttcctttgttccctaagtccaactactaaactgggggatattatgaagggccttgagcatctggattctgcctaataaaaaacatttattttcattgcaaaaaaaaaaaaaaaaaaaaaaaaaaaaaaaaaaaaaaaaaaaaaaaaaaaaaaaaaaaaaaaaaaaaaa

SEQ ID NO: 38 - DNA, 587 bp, synthetic construct
  source 1..587: mol_type = other DNA
taatacgactcactatagggataatacatttgcttctgacacaactgtgttcactagcaacctcaatggcggcccccggcagcgcccggcgacccctgctgctgctactgctgttgctgctgctcggcctcatgcattgtgcgtcagcagcaatggaccctggtcacgcttcttttgtcatggcgtatatccaagaacggttgaaagtgaataccaaactcttggacggtatttccgaatgtctgactacacaattgtgcttcctgtgattggggccatcgtggttggtcgattggggccatcgtggttggtctctgccttatgggtatgggtgtctataaaatccgcctaaggtgtcaatcatctggataccagagaatctaaagctcgctttcttgctgtccaatttctattaaaggttcctttgttccctaagtccaactactaaactgggggatattatgaagggccttgagcatctggattctgcctaataaaaaacatttattttcattgcaaaaaaaaaaaaaaaaaaaaaaaaaaaaaaaaaaaaaaaaaaaaaaaaaaaaaaaaaaaaaaaaaaaaaa

SEQ ID NO: 39 - DNA, 587 bp, synthetic construct
  source 1..587: mol_type = other DNA
taatacgactcactatagggataatacatttgcttctgacacaactgtgttcactagcaacctcaatggcggcccccggcagcgcccggcgacccctgctgctgctactgctgttgctgctgctcggcctcatgcattgtgcgtcagcagcaatggacaaggatgtaatagagtcagtgaaggccttgagcatcaatcgatataccctgtttggtgctcagatgcatgaacctttgggctgtctgactacacaattgtgcttcctgtgattggggccatcgtggttggtcgattggggccatcgtggttggtctctgccttatgggtatgggtgtctataaaatccgcctaaggtgtcaatcatctggataccagagaatctaaagctcgctttcttgctgtccaatttctattaaaggttcctttgttccctaagtccaactactaaactgggggatattatgaagggccttgagcatctggattctgcctaataaaaaacatttattttcattgcaaaaaaaaaaaaaaaaaaaaaaaaaaaaaaaaaaaaaaaaaaaaaaaaaaaaaaaaaaaaaaaaaaaaaa

SEQ ID NO: 40 - DNA, 587 bp, synthetic construct
  source 1..587: mol_type = other DNA
taatacgactcactatagggataatacatttgcttctgacacaactgtgttcactagcaacctcaatggcggcccccggcagcgcccggcgacccctgctgctgctactgctgttgctgctgctcggcctcatgcattgtgcgtcagcagcaatggaccagcacgtgcgggccataaagaagttcgaaatcctgatgtactcctccggcaacacacccgtggagggggcccttctcgactgtctgactacacaattgtgcttcctgtgattggggccatcgtggttggtcgattggggccatcgtggttggtctctgccttatgggtatgggtgtctataaaatccgcctaaggtgtcaatcatctggataccagagaatctaaagctcgctttcttgctgtccaatttctattaaaggttcctttgttccctaagtccaactactaaactgggggatattatgaagggccttgagcatctggattctgcctaataaaaaacatttattttcattgcaaaaaaaaaaaaaaaaaaaaaaaaaaaaaaaaaaaaaaaaaaaaaaaaaaaaaaaaaaaaaaaaaaaaaa

SEQ ID NO: 41 - DNA, 587 bp, synthetic construct
  source 1..587: mol_type = other DNA
taatacgactcactatagggataatacatttgcttctgacacaactgtgttcactagcaacctcaatggcggcccccggcagcgcccggcgacccctgctgctgctactgctgttgctgctgctcggcctcatgcattgtgcgtcagcagcaatggacggggtctcaactgatcgcattaaaatggagcaatatcttctctttgaaagtaacggcaaacacttggttattcccgcagcatgtctgactacacaattgtgcttcctgtgattggggccatcgtggttggtcgattggggccatcgtggttggtctctgccttatgggtatgggtgtctataaaatccgcctaaggtgtcaatcatctggataccagagaatctaaagctcgctttcttgctgtccaatttctattaaaggttcctttgttccctaagtccaactactaaactgggggatattatgaagggccttgagcatctggattctgcctaataaaaaacatttattttcattgcaaaaaaaaaaaaaaaaaaaaaaaaaaaaaaaaaaaaaaaaaaaaaaaaaaaaaaaaaaaaaaaaaaaaaa

SEQ ID NO: 42 - DNA, 587 bp, synthetic construct
  source 1..587: mol_type = other DNA
taatacgactcactatagggataatacatttgcttctgacacaactgtgttcactagcaacctcaatggcggcccccggcagcgcccggcgacccctgctgctgctactgctgttgctgctgctcggcctcatgcattgtgcgtcagcagcaatggacacaataaaggattactctaggagccatttgaaggggatgcccctcttcgctgtcatcgtactggagcaggagaacgcggggtgtctgactacacaattgtgcttcctgtgattggggccatcgtggttggtcgattggggccatcgtggttggtctctgccttatgggtatgggtgtctataaaatccgcctaaggtgtcaatcatctggataccagagaatctaaagctcgctttcttgctgtccaatttctattaaaggttcctttgttccctaagtccaactactaaactgggggatattatgaagggccttgagcatctggattctgcctaataaaaaacatttattttcattgcaaaaaaaaaaaaaaaaaaaaaaaaaaaaaaaaaaaaaaaaaaaaaaaaaaaaaaaaaaaaaaaaaaaaaa

SEQ ID NO: 43 - DNA, 587 bp, synthetic construct
  source 1..587: mol_type = other DNA
taatacgactcactatagggataatacatttgcttctgacacaactgtgttcactagcaacctcaatggcggcccccggcagcgcccggcgacccctgctgctgctactgctgttgctgctgctcggcctcatgcattgtgcgtcagcagcaatggacatgatagagcaagatgttgcggaaattggtctgcgactcgcctataaggtgtccagccctactctccactttaacggtaagtgtctgactacacaattgtgcttcctgtgattggggccatcgtggttggtcgattggggccatcgtggttggtctctgccttatgggtatgggtgtctataaaatccgcctaaggtgtcaatcatctggataccagagaatctaaagctcgctttcttgctgtccaatttctattaaaggttcctttgttccctaagtccaactactaaactgggggatattatgaagggccttgagcatctggattctgcctaataaaaaacatttattttcattgcaaaaaaaaaaaaaaaaaaaaaaaaaaaaaaaaaaaaaaaaaaaaaaaaaaaaaaaaaaaaaaaaaaaaaa

SEQ ID NO: 44 - DNA, 587 bp, synthetic construct
  source 1..587: mol_type = other DNA
taatacgactcactatagggataatacatttgcttctgacacaactgtgttcactagcaacctcaatggcggcccccggcagcgcccggcgacccctgctgctgctactgctgttgctgctgctcggcctcatgcattgtgcgtcagcagcaatggactacaaattgcagaggcatatcgacaaagaaggtacaaatcttgggttcatggttgcccttcccgagtctgtgatagcaagttgtctgactacacaattgtgcttcctgtgattggggccatcgtggttggtcgattggggccatcgtggttggtctctgccttatgggtatgggtgtctataaaatccgcctaaggtgtcaatcatctggataccagagaatctaaagctcgctttcttgctgtccaatttctattaaaggttcctttgttccctaagtccaactactaaactgggggatattatgaagggccttgagcatctggattctgcctaataaaaaacatttattttcattgcaaaaaaaaaaaaaaaaaaaaaaaaaaaaaaaaaaaaaaaaaaaaaaaaaaaaaaaaaaaaaaaaaaaaaa

SEQ ID NO: 45 - DNA, 587 bp, synthetic construct
  source 1..587: mol_type = other DNA
taatacgactcactatagggataatacatttgcttctgacacaactgtgttcactagcaacctcaatggcggcccccggcagcgcccggcgacccctgctgctgctactgctgttgctgctgctcggcctcatgcattgtgcgtcagcagcaatggacataatgcacgcagtacaaaaaacacttattctgcgggaacccaagaacgacctcagctacggggaggggagtgcagtattctgtctgactacacaattgtgcttcctgtgattggggccatcgtggttggtcgattggggccatcgtggttggtctctgccttatgggtatgggtgtctataaaatccgcctaaggtgtcaatcatctggataccagagaatctaaagctcgctttcttgctgtccaatttctattaaaggttcctttgttccctaagtccaactactaaactgggggatattatgaagggccttgagcatctggattctgcctaataaaaaacatttattttcattgcaaaaaaaaaaaaaaaaaaaaaaaaaaaaaaaaaaaaaaaaaaaaaaaaaaaaaaaaaaaaaaaaaaaaaa

SEQ ID NO: 46 - DNA, 587 bp, synthetic construct
  source 1..587: mol_type = other DNA
taatacgactcactatagggataatacatttgcttctgacacaactgtgttcactagcaacctcaatggcggcccccggcagcgcccggcgacccctgctgctgctactgctgttgctgctgctcggcctcatgcattgtgcgtcagcagcaatggacaaggccccggcagaaaatatgacgaaatactcaggtcatagaggggtcagcgaactttttcaagacgtcctgatactcatttgtctgactacacaattgtgcttcctgtgattggggccatcgtggttggtcgattggggccatcgtggttggtctctgccttatgggtatgggtgtctataaaatccgcctaaggtgtcaatcatctggataccagagaatctaaagctcgctttcttgctgtccaatttctattaaaggttcctttgttccctaagtccaactactaaactgggggatattatgaagggccttgagcatctggattctgcctaataaaaaacatttattttcattgcaaaaaaaaaaaaaaaaaaaaaaaaaaaaaaaaaaaaaaaaaaaaaaaaaaaaaaaaaaaaaaaaaaaaaa

SEQ ID NO: 47 - DNA, 587 bp, synthetic construct
  source 1..587: mol_type = other DNA
taatacgactcactatagggataatacatttgcttctgacacaactgtgttcactagcaacctcaatggcggcccccggcagcgcccggcgacccctgctgctgctactgctgttgctgctgctcggcctcatgcattgtgcgtcagcagcaatggacgccgtttcccatctcggcgaaagatatcaaggaaccgccaaaatcatgagtcctttgctgtttaataaggacgttgagatctgtctgactacacaattgtgcttcctgtgattggggccatcgtggttggtcgattggggccatcgtggttggtctctgccttatgggtatgggtgtctataaaatccgcctaaggtgtcaatcatctggataccagagaatctaaagctcgctttcttgctgtccaatttctattaaaggttcctttgttccctaagtccaactactaaactgggggatattatgaagggccttgagcatctggattctgcctaataaaaaacatttattttcattgcaaaaaaaaaaaaaaaaaaaaaaaaaaaaaaaaaaaaaaaaaaaaaaaaaaaaaaaaaaaaaaaaaaaaaa

SEQ ID NO: 48 - DNA, 587 bp, synthetic construct
  source 1..587: mol_type = other DNA
taatacgactcactatagggataatacatttgcttctgacacaactgtgttcactagcaacctcaatggcggcccccggcagcgcccggcgacccctgctgctgctactgctgttgctgctgctcggcctcatgcattgtgcgtcagcagcaatggacgagcccgcactcgacacattggagtatatgagtcttcacaaaggtaaaaacgtcttccaaagtgcgggcatccgcgtgatatgtctgactacacaattgtgcttcctgtgattggggccatcgtggttggtcgattggggccatcgtggttggtctctgccttatgggtatgggtgtctataaaatccgcctaaggtgtcaatcatctggataccagagaatctaaagctcgctttcttgctgtccaatttctattaaaggttcctttgttccctaagtccaactactaaactgggggatattatgaagggccttgagcatctggattctgcctaataaaaaacatttattttcattgcaaaaaaaaaaaaaaaaaaaaaaaaaaaaaaaaaaaaaaaaaaaaaaaaaaaaaaaaaaaaaaaaaaaaaa

SEQ ID NO: 49 - DNA, 587 bp, synthetic construct
  source 1..587: mol_type = other DNA
taatacgactcactatagggataatacatttgcttctgacacaactgtgttcactagcaacctcaatggcggcccccggcagcgcccggcgacccctgctgctgctactgctgttgctgctgctcggcctcatgcattgtgcgtcagcagcaatggacttcgatatgaacaaaaaattgatccaccagtatgagacaccctccgccggtatccgcttggtcgtagaggggtcagcgctttgtctgactacacaattgtgcttcctgtgattggggccatcgtggttggtcgattggggccatcgtggttggtctctgccttatgggtatgggtgtctataaaatccgcctaaggtgtcaatcatctggataccagagaatctaaagctcgctttcttgctgtccaatttctattaaaggttcctttgttccctaagtccaactactaaactgggggatattatgaagggccttgagcatctggattctgcctaataaaaaacatttattttcattgcaaaaaaaaaaaaaaaaaaaaaaaaaaaaaaaaaaaaaaaaaaaaaaaaaaaaaaaaaaaaaaaaaaaaaa

SEQ ID NO: 50 - DNA, 587 bp, synthetic construct
  source 1..587: mol_type = other DNA
taatacgactcactatagggataatacatttgcttctgacacaactgtgttcactagcaacctcaatggcggcccccggcagcgcccggcgacccctgctgctgctactgctgttgctgctgctcggcctcatgcattgtgcgtcagcagcaatggacgtgaacgagcaagtgtccctccgcggatcctacttcaccgcgaaggcgcatatgctggacatcatagaacttggaccgaaatgtctgactacacaattgtgcttcctgtgattggggccatcgtggttggtcgattggggccatcgtggttggtctctgccttatgggtatgggtgtctataaaatccgcctaaggtgtcaatcatctggataccagagaatctaaagctcgctttcttgctgtccaatttctattaaaggttcctttgttccctaagtccaactactaaactgggggatattatgaagggccttgagcatctggattctgcctaataaaaaacatttattttcattgcaaaaaaaaaaaaaaaaaaaaaaaaaaaaaaaaaaaaaaaaaaaaaaaaaaaaaaaaaaaaaaaaaaaaaa

SEQ ID NO: 51 - DNA, 587 bp, synthetic construct
  source 1..587: mol_type = other DNA
taatacgactcactatagggataatacatttgcttctgacacaactgtgttcactagcaacctcaatggcggcccccggcagcgcccggcgacccctgctgctgctactgctgttgctgctgctcggcctcatgcattgtgcgtcagcagcaatggacttgccacaattgggtaaaatattcgggcgaatgaatactaaggcagatgcattgtctgagatagaggtgtatcactctgtttgtctgactacacaattgtgcttcctgtgattggggccatcgtggttggtcgattggggccatcgtggttggtctctgccttatgggtatgggtgtctataaaatccgcctaaggtgtcaatcatctggataccagagaatctaaagctcgctttcttgctgtccaatttctattaaaggttcctttgttccctaagtccaactactaaactgggggatattatgaagggccttgagcatctggattctgcctaataaaaaacatttattttcattgcaaaaaaaaaaaaaaaaaaaaaaaaaaaaaaaaaaaaaaaaaaaaaaaaaaaaaaaaaaaaaaaaaaaaaa

SEQ ID NO: 52 - DNA, 587 bp, synthetic construct
  source 1..587: mol_type = other DNA
taatacgactcactatagggataatacatttgcttctgacacaactgtgttcactagcaacctcaatggcggcccccggcagcgcccggcgacccctgctgctgctactgctgttgctgctgctcggcctcatgcattgtgcgtcagcagcaatggacaaggaccgagcggaggctagcaagataccacaccttctccttgtaatgggtgagtttatcactcagtataatgtcggatcttgtctgactacacaattgtgcttcctgtgattggggccatcgtggttggtcgattggggccatcgtggttggtctctgccttatgggtatgggtgtctataaaatccgcctaaggtgtcaatcatctggataccagagaatctaaagctcgctttcttgctgtccaatttctattaaaggttcctttgttccctaagtccaactactaaactgggggatattatgaagggccttgagcatctggattctgcctaataaaaaacatttattttcattgcaaaaaaaaaaaaaaaaaaaaaaaaaaaaaaaaaaaaaaaaaaaaaaaaaaaaaaaaaaaaaaaaaaaaaa

SEQ ID NO: 53 - DNA, 587 bp, synthetic construct
  source 1..587: mol_type = other DNA
taatacgactcactatagggataatacatttgcttctgacacaactgtgttcactagcaacctcaatggcggcccccggcagcgcccggcgacccctgctgctgctactgctgttgctgctgctcggcctcatgcattgtgcgtcagcagcaatggacgaaggtgtatttgagatgaaacgaaagggtatccaagcactcaacgcgtcagatccgcactacatacttgttttgacgagttgtctgactacacaattgtgcttcctgtgattggggccatcgtggttggtcgattggggccatcgtggttggtctctgccttatgggtatgggtgtctataaaatccgcctaaggtgtcaatcatctggataccagagaatctaaagctcgctttcttgctgtccaatttctattaaaggttcctttgttccctaagtccaactactaaactgggggatattatgaagggccttgagcatctggattctgcctaataaaaaacatttattttcattgcaaaaaaaaaaaaaaaaaaaaaaaaaaaaaaaaaaaaaaaaaaaaaaaaaaaaaaaaaaaaaaaaaaaaaa

SEQ ID NO: 54 - DNA, 587 bp, synthetic construct
  source 1..587: mol_type = other DNA
taatacgactcactatagggataatacatttgcttctgacacaactgtgttcactagcaacctcaatggcggcccccggcagcgcccggcgacccctgctgctgctactgctgttgctgctgctcggcctcatgcattgtgcgtcagcagcaatggacatgaaactcggaaaagtacatgagcagtctccgcttataaaccttataacagcctcacgctttgcaggggactatgtggaatgtctgactacacaattgtgcttcctgtgattggggccatcgtggttggtcgattggggccatcgtggttggtctctgccttatgggtatgggtgtctataaaatccgcctaaggtgtcaatcatctggataccagagaatctaaagctcgctttcttgctgtccaatttctattaaaggttcctttgttccctaagtccaactactaaactgggggatattatgaagggccttgagcatctggattctgcctaataaaaaacatttattttcattgcaaaaaaaaaaaaaaaaaaaaaaaaaaaaaaaaaaaaaaaaaaaaaaaaaaaaaaaaaaaaaaaaaaaaaa

SEQ ID NO: 55 - DNA, 587 bp, synthetic construct
  source 1..587: mol_type = other DNA
taatacgactcactatagggataatacatttgcttctgacacaactgtgttcactagcaacctcaatggcggcccccggcagcgcccggcgacccctgctgctgctactgctgttgctgctgctcggcctcatgcattgtgcgtcagcagcaatggacttgctccacataggggacctcaaaaagatgaactttcaggcaaggggcgctgttgagtacagtacatctgtcattgagccgtgtctgactacacaattgtgcttcctgtgattggggccatcgtggttggtcgattggggccatcgtggttggtctctgccttatgggtatgggtgtctataaaatccgcctaaggtgtcaatcatctggataccagagaatctaaagctcgctttcttgctgtccaatttctattaaaggttcctttgttccctaagtccaactactaaactgggggatattatgaagggccttgagcatctggattctgcctaataaaaaacatttattttcattgcaaaaaaaaaaaaaaaaaaaaaaaaaaaaaaaaaaaaaaaaaaaaaaaaaaaaaaaaaaaaaaaaaaaaaa

SEQ ID NO: 56 - DNA, 587 bp, synthetic construct
  source 1..587: mol_type = other DNA
taatacgactcactatagggataatacatttgcttctgacacaactgtgttcactagcaacctcaatggcggcccccggcagcgcccggcgacccctgctgctgctactgctgttgctgctgctcggcctcatgcattgtgcgtcagcagcaatggacaaacactttcgaatacccgtggccaacaccggaggggacgtgctgctttctgagaagatgagtgcgtatgagctcattcaatgtctgactacacaattgtgcttcctgtgattggggccatcgtggttggtcgattggggccatcgtggttggtctctgccttatgggtatgggtgtctataaaatccgcctaaggtgtcaatcatctggataccagagaatctaaagctcgctttcttgctgtccaatttctattaaaggttcctttgttccctaagtccaactactaaactgggggatattatgaagggccttgagcatctggattctgcctaataaaaaacatttattttcattgcaaaaaaaaaaaaaaaaaaaaaaaaaaaaaaaaaaaaaaaaaaaaaaaaaaaaaaaaaaaaaaaaaaaaaa

SEQ ID NO: 57 - DNA, 587 bp, synthetic construct
  source 1..587: mol_type = other DNA
taatacgactcactatagggataatacatttgcttctgacacaactgtgttcactagcaacctcaatggcggcccccggcagcgcccggcgacccctgctgctgctactgctgttgctgctgctcggcctcatgcattgtgcgtcagcagcaatggacctgtataagatgaggaagctggacgaggctgaactgtttatcggcggtataacgaacccatccgccgtgcatgtacagagctgtctgactacacaattgtgcttcctgtgattggggccatcgtggttggtcgattggggccatcgtggttggtctctgccttatgggtatgggtgtctataaaatccgcctaaggtgtcaatcatctggataccagagaatctaaagctcgctttcttgctgtccaatttctattaaaggttcctttgttccctaagtccaactactaaactgggggatattatgaagggccttgagcatctggattctgcctaataaaaaacatttattttcattgcaaaaaaaaaaaaaaaaaaaaaaaaaaaaaaaaaaaaaaaaaaaaaaaaaaaaaaaaaaaaaaaaaaaaaa

SEQ ID NO: 58 - DNA, 587 bp, synthetic construct
  source 1..587: mol_type = other DNA
taatacgactcactatagggataatacatttgcttctgacacaactgtgttcactagcaacctcaatggcggcccccggcagcgcccggcgacccctgctgctgctactgctgttgctgctgctcggcctcatgcattgtgcgtcagcagcaatggacctgaatattgtatacccccagatgcgcaaaatagaggatgcgaagacctctttgagcgaggcgtttctggggggacacgtctgtctgactacacaattgtgcttcctgtgattggggccatcgtggttggtcgattggggccatcgtggttggtctctgccttatgggtatgggtgtctataaaatccgcctaaggtgtcaatcatctggataccagagaatctaaagctcgctttcttgctgtccaatttctattaaaggttcctttgttccctaagtccaactactaaactgggggatattatgaagggccttgagcatctggattctgcctaataaaaaacatttattttcattgcaaaaaaaaaaaaaaaaaaaaaaaaaaaaaaaaaaaaaaaaaaaaaaaaaaaaaaaaaaaaaaaaaaaaaa

SEQ ID NO: 59 - DNA, 587 bp, synthetic construct
  source 1..587: mol_type = other DNA
taatacgactcactatagggataatacatttgcttctgacacaactgtgttcactagcaacctcaatggcggcccccggcagcgcccggcgacccctgctgctgctactgctgttgctgctgctcggcctcatgcattgtgcgtcagcagcaatggacgggaaggaagagatcatcttgtcttcagataacggatatgctttcaaaaggttgcatatgcctcaactcgtaacagtggcatgtctgactacacaattgtgcttcctgtgattggggccatcgtggttggtcgattggggccatcgtggttggtctctgccttatgggtatgggtgtctataaaatccgcctaaggtgtcaatcatctggataccagagaatctaaagctcgctttcttgctgtccaatttctattaaaggttcctttgttccctaagtccaactactaaactgggggatattatgaagggccttgagcatctggattctgcctaataaaaaacatttattttcattgcaaaaaaaaaaaaaaaaaaaaaaaaaaaaaaaaaaaaaaaaaaaaaaaaaaaaaaaaaaaaaaaaaaaaaa

SEQ ID NO: 60 - DNA, 587 bp, synthetic construct
  source 1..587: mol_type = other DNA
taatacgactcactatagggataatacatttgcttctgacacaactgtgttcactagcaacctcaatggcggcccccggcagcgcccggcgacccctgctgctgctactgctgttgctgctgctcggcctcatgcattgtgcgtcagcagcaatggacgatttcagtgagggaggattgtataacgctcagaaagagaaaccacttgcagtgattcttcatagggtgatgtctacaatctgtctgactacacaattgtgcttcctgtgattggggccatcgtggttggtcgattggggccatcgtggttggtctctgccttatgggtatgggtgtctataaaatccgcctaaggtgtcaatcatctggataccagagaatctaaagctcgctttcttgctgtccaatttctattaaaggttcctttgttccctaagtccaactactaaactgggggatattatgaagggccttgagcatctggattctgcctaataaaaaacatttattttcattgcaaaaaaaaaaaaaaaaaaaaaaaaaaaaaaaaaaaaaaaaaaaaaaaaaaaaaaaaaaaaaaaaaaaaaa

SEQ ID NO: 61 - DNA, 587 bp, synthetic construct
  source 1..587: mol_type = other DNA
taatacgactcactatagggataatacatttgcttctgacacaactgtgttcactagcaacctcaatggcggcccccggcagcgcccggcgacccctgctgctgctactgctgttgctgctgctcggcctcatgcattgtgcgtcagcagcaatggactcccacgccaaggaggttgctacgggctcattgatccagtttagactgggtgagccgatggacatttataaggttcttaactgtctgactacacaattgtgcttcctgtgattggggccatcgtggttggtcgattggggccatcgtggttggtctctgccttatgggtatgggtgtctataaaatccgcctaaggtgtcaatcatctggataccagagaatctaaagctcgctttcttgctgtccaatttctattaaaggttcctttgttccctaagtccaactactaaactgggggatattatgaagggccttgagcatctggattctgcctaataaaaaacatttattttcattgcaaaaaaaaaaaaaaaaaaaaaaaaaaaaaaaaaaaaaaaaaaaaaaaaaaaaaaaaaaaaaaaaaaaaaa

SEQ ID NO: 62 - protein, 31 aa, synthetic construct
MAAPGSARRPLLLLLLLLLLGLMHCASAAMD

SEQ ID NO: 63 - protein, 40 aa, synthetic construct
SSDYTIVLPVIGAIVVGLCLMGMGVYKIRLRCQSSGYQRI